European Patent Application EP 4 286 520 A1, published December 6, 2023. Title: ANTIGEN BINDING PROTEIN AND USE THEREOF. Applicant: MINGHUI PHARMACEUTICAL (HANGZHOU) LIMITED; MINGHUI PHARMACEUTICAL (SHANGHAI) LIMITED. The sequence listing filed with the application follows.

SEQUENCE LISTING (236 sequences)

SEQ ID NO: 1 - protein, 8 aa, Artificial Sequence
  MHPD1-A+1 HCDR1
GSDPSIYA

SEQ ID NO: 2 - protein, 8 aa, Artificial Sequence
  MHPD1-A HCDR2
IGWSAATT

SEQ ID NO: 3 - protein, 11 aa, Artificial Sequence
  MHPD1-A+2-17+20-21+23+27-29+32-33+35-36+39+41-42+44-45+47 HCDR3
AADLDHSGFDY

SEQ ID NO: 4 - protein, 8 aa, Artificial Sequence
  MHPD1-A-2 HCDR1
GRFPSIYA

SEQ ID NO: 5 - protein, 8 aa, Artificial Sequence
  MHPD1-A-3 HCDR1
GSGRSIYA

SEQ ID NO: 6 - protein, 8 aa, Artificial Sequence
  MHPD1-A-4 HCDR1
GSVGSIYA

SEQ ID NO: 7 - protein, 8 aa, Artificial Sequence
  MHPD1-A-5 HCDR1
GSSLSIYA

SEQ ID NO: 8 - protein, 8 aa, Artificial Sequence
  MHPD1-A-6 HCDR1
GRRPSIYA

SEQ ID NO: 9 - protein, 8 aa, Artificial Sequence
  MHPD1-A-7+21-22+31+39-40+43+48-49 HCDR1
GSRRSIYA

SEQ ID NO: 10 - protein, 8 aa, Artificial Sequence
  MHPD1-A-8 HCDR1
GGRPSIYA

SEQ ID NO: 11 - protein, 8 aa, Artificial Sequence
  MHPD1-A-9 HCDR1
GSGHSIYA

SEQ ID NO: 12 - protein, 8 aa, Artificial Sequence
  MHPD1-A-10 HCDR1
GSDDRIYA

SEQ ID NO: 13 - protein, 8 aa, Artificial Sequence
  MHPD1-A-11 HCDR1
GSQLSIYA

SEQ ID NO: 14 - protein, 8 aa, Artificial Sequence
  MHPD1-A-12 HCDR1
GSDYAIYA

SEQ ID NO: 15 - protein, 8 aa, Artificial Sequence
  MHPD1-A-13 HCDR1
HADPSIYA

SEQ ID NO: 16 - protein, 8 aa, Artificial Sequence
  MHPD1-A-14 HCDR1
SHRPSIYA

SEQ ID NO: 17 - protein, 8 aa, Artificial Sequence
  MHPD1-A-15 HCDR1
GLRRSIYA

SEQ ID NO: 18 - protein, 8 aa, Artificial Sequence
  MHPD1-A-16 HCDR1
GSRVSIYA

SEQ ID NO: 19 - protein, 8 aa, Artificial Sequence
  MHPD1-A-17 HCDR1
GSISSIYA

SEQ ID NO: 20 - protein, 8 aa, Artificial Sequence
  MHPD1-A-18 HCDR1
GSRSSIYA

SEQ ID NO: 21 - protein, 8 aa, Artificial Sequence
  MHPD1-A-19 HCDR1
GSEVSIYA

SEQ ID NO: 22 - protein, 8 aa, Artificial Sequence
  MHPD1-A-20 HCDR1
GSRKSIYA

SEQ ID NO: 23 - protein, 8 aa, Artificial Sequence
  MHPD1-A-23 HCDR1
GTRRSIYA

SEQ ID NO: 24 - protein, 8 aa, Artificial Sequence
  MHPD1-A-24 HCDR1
GSRHSIYA

SEQ ID NO: 25 - protein, 8 aa, Artificial Sequence
  MHPD1-A-25+30 HCDR1
GVRRSIYA

SEQ ID NO: 26 - protein, 8 aa, Artificial Sequence
  MHPD1-A-26 HCDR1
GSRSNIYA

SEQ ID NO: 27 - protein, 8 aa, Artificial Sequence
  MHPD1-A-27 HCDR1
KSRRSIYA

SEQ ID NO: 28 - protein, 8 aa, Artificial Sequence
  MHPD1-A-28 HCDR1
KLRRSIYA

SEQ ID NO: 29 - protein, 8 aa, Artificial Sequence
  MHPD1-A-29 HCDR1
GSGGSIYA

SEQ ID NO: 30 - protein, 8 aa, Artificial Sequence
  MHPD1-A-32 HCDR1
KNRRSIYA

SEQ ID NO: 31 - protein, 8 aa, Artificial Sequence
  MHPD1-A-33 HCDR1
GSRSQIYA

SEQ ID NO: 32 - protein, 8 aa, Artificial Sequence
  MHPD1-A-35 HCDR1
APRRSIYA

SEQ ID NO: 33 - protein, 8 aa, Artificial Sequence
  MHPD1-A-36 HCDR1
GSRRFIYA

SEQ ID NO: 34 - protein, 8 aa, Artificial Sequence
  MHPD1-A-37 HCDR1
GARRSIYA

SEQ ID NO: 35 - protein, 8 aa, Artificial Sequence
  MHPD1-A-38 HCDR1
GNRRSIYA

SEQ ID NO: 36 - protein, 8 aa, Artificial Sequence
  MHPD1-A-41 HCDR1
VSRRSIYA

SEQ ID NO: 37 - protein, 8 aa, Artificial Sequence
  MHPD1-A-42 HCDR1
GSRQTIYA

SEQ ID NO: 38 - protein, 8 aa, Artificial Sequence
  MHPD1-A-44 HCDR1
GSRTRIYA

SEQ ID NO: 39 - protein, 8 aa, Artificial Sequence
  MHPD1-A-45 HCDR1
HLRRSIYA

SEQ ID NO: 40 - protein, 8 aa, Artificial Sequence
  MHPD1-A-46 HCDR1
GSKGSIYA

SEQ ID NO: 41 - protein, 8 aa, Artificial Sequence
  MHPD1-A-47 HCDR1
GSRLSIYA

SEQ ID NO: 42 - protein, 8 aa, Artificial Sequence
  MHPD1-A-1 HCDR2
IGWAWATT

SEQ ID NO: 43 - protein, 8 aa, Artificial Sequence
  MHPD1-A-2+10+14 HCDR2
IGWRYATT

SEQ ID NO: 44 - protein, 8 aa, Artificial Sequence
  MHPD1-A-3+9 HCDR2
IGWSYATT

SEQ ID NO: 45 - protein, 8 aa, Artificial Sequence
  MHPD1-A-4+8+12 HCDR2
IGWAFATT

SEQ ID NO: 46 - protein, 8 aa, Artificial Sequence
  MHPD1-A-5+7+16-17+19-20+22-27+29+32-33+37-38+40-41+43+45-49 HCDR2
IGWAYATT

SEQ ID NO: 47 - protein, 8 aa, Artificial Sequence
  MHPD1-A-6+13 HCDR2
IGWNYATT

SEQ ID NO: 48 - protein, 8 aa, Artificial Sequence
  MHPD1-A-11 HCDR2
IGWRFATT

SEQ ID NO: 49 - protein, 8 aa, Artificial Sequence
  MHPD1-A-15 HCDR2
IGWAYSTT

SEQ ID NO: 50 - protein, 8 aa, Artificial Sequence
  MHPD1-A-18+31 HCDR2
LGWAYATT

SEQ ID NO: 51 - protein, 8 aa, Artificial Sequence
  MHPD1-A-21 HCDR2
IGWAYATS

SEQ ID NO: 52 - protein, 8 aa, Artificial Sequence
  MHPD1-A-28+30+36+42 HCDR2
IGWAYATQ

SEQ ID NO: 53 - protein, 8 aa, Artificial Sequence
  MHPD1-A-35 HCDR2
IGWAYGTT

SEQ ID NO: 54 - protein, 8 aa, Artificial Sequence
  MHPD1-A-39+44 HCDR2
IGWAYATE

SEQ ID NO: 55 - protein, 11 aa, Artificial Sequence
  MHPD1-A-1+46 HCDR3
AADLDRSGFDY

SEQ ID NO: 56 - protein, 11 aa, Artificial Sequence
  MHPD1-A-18 HCDR3
AADLDHLGFDY

SEQ ID NO: 57 - protein, 11 aa, Artificial Sequence
  MHPD1-A-19+38 HCDR3
AADLDRRGFDY

SEQ ID NO: 58 - protein, 11 aa, Artificial Sequence
  MHPD1-A-22 HCDR3
AADLDRGGFDY

SEQ ID NO: 59 - protein, 11 aa, Artificial Sequence
  MHPD1-A-24+43 HCDR3
AADLDRAGFDY

SEQ ID NO: 60 - protein, 11 aa, Artificial Sequence
  MHPD1-A-25 HCDR3
AADLDRHGFDY

SEQ ID NO: 61 - protein, 11 aa, Artificial Sequence
  MHPD1-A-26 HCDR3
AADLDRDGFDY

SEQ ID NO: 62 - protein, 11 aa, Artificial Sequence
  MHPD1-A-30 HCDR3
AADIDHSGFDY

SEQ ID NO: 63 - protein, 11 aa, Artificial Sequence
  MHPD1-A-31 HCDR3
AADLDHHGFDY

SEQ ID NO: 64 - protein, 11 aa, Artificial Sequence
  MHPD1-A-37 HCDR3
AADLDRTGFDY

SEQ ID NO: 65 - protein, 11 aa, Artificial Sequence
  MHPD1-A-40 HCDR3
AADLDVAGFDY

SEQ ID NO: 66 - protein, 11 aa, Artificial Sequence
  MHPD1-A-48 HCDR3
AADLDRNGFDY

SEQ ID NO: 67 - protein, 11 aa, Artificial Sequence
  MHPD1-A-49 HCDR3
AADLDRVGFDY

SEQ ID NO: 68 - protein, 25 aa, Artificial Sequence
  H-FR1 of antibody+MHPD1-A-H3+5-8 H-FR1
QVQLVESGGGSVQVGGSLTLSCAAS

SEQ ID NO: 69 - protein, 17 aa, Artificial Sequence
  H-FR2 of antibody +MHPD1-A-H1-3+5+9-10+12+14-16 H-FR2
MGWFRQAPGKEHEFVAG

SEQ ID NO: 70 - protein, 38 aa, Artificial Sequence
  H-FR3 of antibody +MHPD1-A-H1+6+8 H-FR3
YYADSVKGRFGISRDNTKNTVALLMNSLKPEDTAIYYC

SEQ ID NO: 71 - protein, 11 aa, Artificial Sequence
  H-FR4 of antibody +MHPD1-A-H2-3+5-8 H-FR4
WGQGTQVTVSS

SEQ ID NO: 72 - protein, 118 aa, Artificial Sequence
  MHPD1-A
QVQLVESGGGSVQVGGSLTLSCAASGSDPSIYAMGWFRQAPGKEHEFVAGIGWSAATTYYADSVKGRFGISRDNTKNTVALLMNSLKPEDTAIYYCAADLDHSGFDYWGQGTQVTVSS

SEQ ID NO: 73 - protein, 118 aa, Artificial Sequence
  MHPD1-A-1
QVQLVESGGGSVQVGGSLTLSCAASGSDPSIYAMGWFRQAPGKEHEFVAGIGWAWATTYYADSVKGRFGISRDNTKNTVALLMNSLKPEDTAIYYCAADLDRSGFDYWGQGTQVTVSS

SEQ ID NO: 74 - protein, 118 aa, Artificial Sequence
  MHPD1-A-2
QVQLVESGGGSVQVGGSLTLSCAASGRFPSIYAMGWFRQAPGKEHEFVAGIGWRYATTYYADSVKGRFGISRDNTKNTVALLMNSLKPEDTAIYYCAADLDHSGFDYWGQGTQVTVSS

SEQ ID NO: 75 - protein, 118 aa, Artificial Sequence
  MHPD1-A-3
QVQLVESGGGSVQVGGSLTLSCAASGSGRSIYAMGWFRQAPGKEHEFVAGIGWSYATTYYADSVKGRFGISRDNTKNTVALLMNSLKPEDTAIYYCAADLDHSGFDYWGQGTQVTVSS

SEQ ID NO: 76 - protein, 118 aa, Artificial Sequence
  MHPD1-A-4
QVQLVESGGGSVQVGGSLTLSCAASGSVGSIYAMGWFRQAPGKEHEFVAGIGWAFATTYYADSVKGRFGISRDNTKNTVALLMNSLKPEDTAIYYCAADLDHSGFDYWGQGTQVTVSS

SEQ ID NO: 77 - protein, 118 aa, Artificial Sequence
  MHPD1-A-5
QVQLVESGGGSVQVGGSLTLSCAASGSSLSIYAMGWFRQAPGKEHEFVAGIGWAYATTYYADSVKGRFGISRDNTKNTVALLMNSLKPEDTAIYYCAADLDHSGFDYWGQGTQVTVSS

SEQ ID NO: 78 - protein, 118 aa, Artificial Sequence
  MHPD1-A-6
QVQLVESGGGSVQVGGSLTLSCAASGRRPSIYAMGWFRQAPGKEHEFVAGIGWNYATTYYADSVKGRFGISRDNTKNTVALLMNSLKPEDTAIYYCAADLDHSGFDYWGQGTQVTVSS

SEQ ID NO: 79 - protein, 118 aa, Artificial Sequence
  MHPD1-A-7
QVQLVESGGGSVQVGGSLTLSCAASGSRRSIYAMGWFRQAPGKEHEFVAGIGWAYATTYYADSVKGRFGISRDNTKNTVALLMNSLKPEDTAIYYCAADLDHSGFDYWGQGTQVTVSS

SEQ ID NO: 80 - protein, 118 aa, Artificial Sequence
  MHPD1-A-8
QVQLVESGGGSVQVGGSLTLSCAASGGRPSIYAMGWFRQAPGKEHEFVAGIGWAFATTYYADSVKGRFGISRDNTKNTVALLMNSLKPEDTAIYYCAADLDHSGFDYWGQGTQVTVSS

SEQ ID NO: 81 - protein, 118 aa, Artificial Sequence
  MHPD1-A-9
QVQLVESGGGSVQVGGSLTLSCAASGSGHSIYAMGWFRQAPGKEHEFVAGIGWSYATTYYADSVKGRFGISRDNTKNTVALLMNSLKPEDTAIYYCAADLDHSGFDYWGQGTQVTVSS

SEQ ID NO: 82 - protein, 118 aa, Artificial Sequence
  MHPD1-A-10
QVQLVESGGGSVQVGGSLTLSCAASGSDDRIYAMGWFRQAPGKEHEFVAGIGWRYATTYYADSVKGRFGISRDNTKNTVALLMNSLKPEDTAIYYCAADLDHSGFDYWGQGTQVTVSS

SEQ ID NO: 83 - protein, 118 aa, Artificial Sequence
  MHPD1-A-11
QVQLVESGGGSVQVGGSLTLSCAASGSQLSIYAMGWFRQAPGKEHEFVAGIGWRFATTYYADSVKGRFGISRDNTKNTVALLMNSLKPEDTAIYYCAADLDHSGFDYWGQGTQVTVSS

SEQ ID NO: 84 - protein, 118 aa, Artificial Sequence
  MHPD1-A-12
QVQLVESGGGSVQVGGSLTLSCAASGSDYAIYAMGWFRQAPGKEHEFVAGIGWAFATTYYADSVKGRFGISRDNTKNTVALLMNSLKPEDTAIYYCAADLDHSGFDYWGQGTQVTVSS

SEQ ID NO: 85 - protein, 118 aa, Artificial Sequence
  MHPD1-A-13
QVQLVESGGGSVQVGGSLTLSCAASHADPSIYAMGWFRQAPGKEHEFVAGIGWNYATTYYADSVKGRFGISRDNTKNTVALLMNSLKPEDTAIYYCAADLDHSGFDYWGQGTQVTVSS

SEQ ID NO: 86 - protein, 118 aa, Artificial Sequence
  MHPD1-A-14
QVQLVESGGGSVQVGGSLTLSCAASSHRPSIYAMGWFRQAPGKEHEFVAGIGWRYATTYYADSVKGRFGISRDNTKNTVALLMNSLKPEDTAIYYCAADLDHSGFDYWGQGTQVTVSS

SEQ ID NO: 87 - protein, 118 aa, Artificial Sequence
  MHPD1-A-15
QVQLVESGGGSVQVGGSLTLSCAASGLRRSIYAMGWFRQAPGKEHEFVAGIGWAYSTTYYADSVKGRFGISRDNTKNTVALLMNSLKPEDTAIYYCAADLDHSGFDYWGQGTQVTVSS

SEQ ID NO: 88 - protein, 118 aa, Artificial Sequence
  MHPD1-A-16
QVQLVESGGGSVQVGGSLTLSCAASGSRVSIYAMGWFRQAPGKEHEFVAGIGWAYATTYYADSVKGRFGISRDNTKNTVALLMNSLKPEDTAIYYCAADLDHSGFDYWGQGTQVTVSS

SEQ ID NO: 89 - protein, 118 aa, Artificial Sequence
  MHPD1-A-17
QVQLVESGGGSVQVGGSLTLSCAASGSISSIYAMGWFRQAPGKEHEFVAGIGWAYATTYYADSVKGRFGISRDNTKNTVALLMNSLKPEDTAIYYCAADLDHSGFDYWGQGTQVTVSS

SEQ ID NO: 90 - protein, 118 aa, Artificial Sequence
  MHPD1-A-18
QVQLVESGGGSVQVGGSLTLSCAASGSRSSIYAMGWFRQAPGKEHEFVAGLGWAYATTYYADSVKGRFGISRDNTKNTVALLMNSLKPEDTAIYYCAADLDHLGFDYWGQGTQVTVSS

SEQ ID NO: 91 - protein, 118 aa, Artificial Sequence
  MHPD1-A-19
QVQLVESGGGSVQVGGSLTLSCAASGSEVSIYAMGWFRQAPGKEHEFVAGIGWAYATTYYADSVKGRFGISRDNTKNTVALLMNSLKPEDTAIYYCAADLDRRGFDYWGQGTQVTVSS

SEQ ID NO: 92 - protein, 118 aa, Artificial Sequence
  MHPD1-A-20
QVQLVESGGGSVQVGGSLTLSCAASGSRKSIYAMGWFRQAPGKEHEFVAGIGWAYATTYYADSVKGRFGISRDNTKNTVALLMNSLKPEDTAIYYCAADLDHSGFDYWGQGTQVTVSS

SEQ ID NO: 93 - protein, 118 aa, Artificial Sequence
  MHPD1-A-21
QVQLVESGGGSVQVGGSLTLSCAASGSRRSIYAMGWFRQAPGKEHEFVAGIGWAYATSYYADSVKGRFGISRDNTKNTVALLMNSLKPEDTAIYYCAADLDHSGFDYWGQGTQVTVSS

SEQ ID NO: 94 - protein, 118 aa, Artificial Sequence
  MHPD1-A-22
QVQLVESGGGSVQVGGSLTLSCAASGSRRSIYAMGWFRQAPGKEHEFVAGIGWAYATTYYADSVKGRFGISRDNTKNTVALLMNSLKPEDTAIYYCAADLDRGGFDYWGQGTQVTVSS

SEQ ID NO: 95 - protein, 118 aa, Artificial Sequence
  MHPD1-A-23
QVQLVESGGGSVQVGGSLTLSCAASGTRRSIYAMGWFRQAPGKEHEFVAGIGWAYATTYYADSVKGRFGISRDNTKNTVALLMNSLKPEDTAIYYCAADLDHSGFDYWGQGTQVTVSS

SEQ ID NO: 96 - protein, 118 aa, Artificial Sequence
  MHPD1-A-24
QVQLVESGGGSVQVGGSLTLSCAASGSRHSIYAMGWFRQAPGKEHEFVAGIGWAYATTYYADSVKGRFGISRDNTKNTVALLMNSLKPEDTAIYYCAADLDRAGFDYWGQGTQVTVSS

SEQ ID NO: 97 - protein, 118 aa, Artificial Sequence
  MHPD1-A-25
QVQLVESGGGSVQVGGSLTLSCAASGVRRSIYAMGWFRQAPGKEHEFVAGIGWAYATTYYADSVKGRFGISRDNTKNTVALLMNSLKPEDTAIYYCAADLDRHGFDYWGQGTQVTVSS

SEQ ID NO: 98 - protein, 118 aa, Artificial Sequence
  MHPD1-A-26
QVQLVESGGGSVQVGGSLTLSCAASGSRSNIYAMGWFRQAPGKEHEFVAGIGWAYATTYYADSVKGRFGISRDNTKNTVALLMNSLKPEDTAIYYCAADLDRDGFDYWGQGTQVTVSS

SEQ ID NO: 99 - protein, 118 aa, Artificial Sequence
  MHPD1-A-27
QVQLVESGGGSVQVGGSLTLSCAASKSRRSIYAMGWFRQAPGKEHEFVAGIGWAYATTYYADSVKGRFGISRDNTKNTVALLMNSLKPEDTAIYYCAADLDHSGFDYWGQGTQVTVSS

SEQ ID NO: 100 - protein, 118 aa, Artificial Sequence
  MHPD1-A-28
QVQLVESGGGSVQVGGSLTLSCAASKLRRSIYAMGWFRQAPGKEHEFVAGIGWAYATQYYADSVKGRFGISRDNTKNTVALLMNSLKPEDTAIYYCAADLDHSGFDYWGQGTQVTVSS

SEQ ID NO: 101 - protein, 118 aa, Artificial Sequence
  MHPD1-A-29
QVQLVESGGGSVQVGGSLTLSCAASGSGGSIYAMGWFRQAPGKEHEFVAGIGWAYATTYYADSVKGRFGISRDNTKNTVALLMNSLKPEDTAIYYCAADLDHSGFDYWGQGTQVTVSS

SEQ ID NO: 102 - protein, 118 aa, Artificial Sequence
  MHPD1-A-30
QVQLVESGGGSVQVGGSLTLSCAASGVRRSIYAMGWFRQAPGKEHEFVAGIGWAYATQYYADSVKGRFGISRDNTKNTVALLMNSLKPEDTAIYYCAADIDHSGFDYWGQGTQVTVSS

SEQ ID NO: 103 - protein, 118 aa, Artificial Sequence
  MHPD1-A-31
QVQLVESGGGSVQVGGSLTLSCAASGSRRSIYAMGWFRQAPGKEHEFVAGLGWAYATTYYADSVKGRFGISRDNTKNTVALLMNSLKPEDTAIYYCAADLDHHGFDYWGQGTQVTVSS

SEQ ID NO: 104 - protein, 118 aa, Artificial Sequence
  MHPD1-A-32
QVQLVESGGGSVQVGGSLTLSCAASKNRRSIYAMGWFRQAPGKEHEFVAGIGWAYATTYYADSVKGRFGISRDNTKNTVALLMNSLKPEDTAIYYCAADLDHSGFDYWGQGTQVTVSS

SEQ ID NO: 105 - protein, 118 aa, Artificial Sequence
  MHPD1-A-33
QVQLVESGGGSVQVGGSLTLSCAASGSRSQIYAMGWFRQAPGKEHEFVAGIGWAYATTYYADSVKGRFGISRDNTKNTVALLMNSLKPEDTAIYYCAADLDHSGFDYWGQGTQVTVSS

SEQ ID NO: 106 - protein, 118 aa, Artificial Sequence
  MHPD1-A-35
QVQLVESGGGSVQVGGSLTLSCAASAPRRSIYAMGWFRQAPGKEHEFVAGIGWAYGTTYYADSVKGRFGISRDNTKNTVALLMNSLKPEDTAIYYCAADLDHSGFDYWGQGTQVTVSS

SEQ ID NO: 107 - protein, 118 aa, Artificial Sequence
  MHPD1-A-36
QVQLVESGGGSVQVGGSLTLSCAASGSRRFIYAMGWFRQAPGKEHEFVAGIGWAYATQYYADSVKGRFGISRDNTKNTVALLMNSLKPEDTAIYYCAADLDHSGFDYWGQGTQVTVSS

SEQ ID NO: 108 - protein, 118 aa, Artificial Sequence
  MHPD1-A-37
QVQLVESGGGSVQVGGSLTLSCAASGARRSIYAMGWFRQAPGKEHEFVAGIGWAYATTYYADSVKGRFGISRDNTKNTVALLMNSLKPEDTAIYYCAADLDRTGFDYWGQGTQVTVSS

SEQ ID NO: 109 - protein, 118 aa, Artificial Sequence
  MHPD1-A-38
QVQLVESGGGSVQVGGSLTLSCAASGNRRSIYAMGWFRQAPGKEHEFVAGIGWAYATTYYADSVKGRFGISRDNTKNTVALLMNSLKPEDTAIYYCAADLDRRGFDYWGQGTQVTVSS

SEQ ID NO: 110 - protein, 118 aa, Artificial Sequence
  MHPD1-A-39
QVQLVESGGGSVQVGGSLTLSCAASGSRRSIYAMGWFRQAPGKEHEFVAGIGWAYATEYYADSVKGRFGISRDNTKNTVALLMNSLKPEDTAIYYCAADLDHSGFDYWGQGTQVTVSS

SEQ ID NO: 111 - protein, 118 aa, Artificial Sequence
  MHPD1-A-40
QVQLVESGGGSVQVGGSLTLSCAASGSRRSIYAMGWFRQAPGKEHEFVAGIGWAYATTYYADSVKGRFGISRDNTKNTVALLMNSLKPEDTAIYYCAADLDVAGFDYWGQGTQVTVSS

SEQ ID NO: 112 - protein, 118 aa, Artificial Sequence
  MHPD1-A-41
QVQLVESGGGSVQVGGSLTLSCAASVSRRSIYAMGWFRQAPGKEHEFVAGIGWAYATTYYADSVKGRFGISRDNTKNTVALLMNSLKPEDTAIYYCAADLDHSGFDYWGQGTQVTVSS

SEQ ID NO: 113 - protein, 118 aa, Artificial Sequence
  MHPD1-A-42
QVQLVESGGGSVQVGGSLTLSCAASGSRQTIYAMGWFRQAPGKEHEFVAGIGWAYATQYYADSVKGRFGISRDNTKNTVALLMNSLKPEDTAIYYCAADLDHSGFDYWGQGTQVTVSS

SEQ ID NO: 114 - protein, 118 aa, Artificial Sequence
  MHPD1-A-43
QVQLVESGGGSVQVGGSLTLSCAASGSRRSIYAMGWFRQAPGKEHEFVAGIGWAYATTYYADSVKGRFGISRDNTKNTVALLMNSLKPEDTAIYYCAADLDRAGFDYWGQGTQVTVSS

SEQ ID NO: 115 - protein, 118 aa, Artificial Sequence
  MHPD1-A-44
QVQLVESGGGSVQVGGSLTLSCAASGSRTRIYAMGWFRQAPGKEHEFVAGIGWAYATEYYADSVKGRFGISRDNTKNTVALLMNSLKPEDTAIYYCAADLDHSGFDYWGQGTQVTVSS

SEQ ID NO: 116 - protein, 118 aa, Artificial Sequence
  MHPD1-A-45
QVQLVESGGGSVQVGGSLTLSCAASHLRRSIYAMGWFRQAPGKEHEFVAGIGWAYATTYYADSVKGRFGISRDNTKNTVALLMNSLKPEDTAIYYCAADLDHSGFDYWGQGTQVTVSS

SEQ ID NO: 117 - protein, 118 aa, Artificial Sequence
  MHPD1-A-46
QVQLVESGGGSVQVGGSLTLSCAASGSKGSIYAMGWFRQAPGKEHEFVAGIGWAYATTYYADSVKGRFGISRDNTKNTVALLMNSLKPEDTAIYYCAADLDRSGFDYWGQGTQVTVSS

SEQ ID NO: 118 - protein, 118 aa, Artificial Sequence
  MHPD1-A-47
QVQLVESGGGSVQVGGSLTLSCAASGSRLSIYAMGWFRQAPGKEHEFVAGIGWAYATTYYADSVKGRFGISRDNTKNTVALLMNSLKPEDTAIYYCAADLDHSGFDYWGQGTQVTVSS

SEQ ID NO: 119 - protein, 118 aa, Artificial Sequence
  MHPD1-A-48
QVQLVESGGGSVQVGGSLTLSCAASGSRRSIYAMGWFRQAPGKEHEFVAGIGWAYATTYYADSVKGRFGISRDNTKNTVALLMNSLKPEDTAIYYCAADLDRNGFDYWGQGTQVTVSS

SEQ ID NO: 120 - protein, 118 aa, Artificial Sequence
  MHPD1-A-49
QVQLVESGGGSVQVGGSLTLSCAASGSRRSIYAMGWFRQAPGKEHEFVAGIGWAYATTYYADSVKGRFGISRDNTKNTVALLMNSLKPEDTAIYYCAADLDRVGFDYWGQGTQVTVSS

SEQ ID NO: 121 - protein, 232 aa, Artificial Sequence
  Fc domain (hIgG1 Fc D239E,L241M)
EPKSCDKTHTCPPCPAPELLGGPSVFLFPPKPKDTLMISRTPEVTCVVVDVSHEDPEVKFNWYVDGVEVHNAKTKPREEQYNSTYRVVSVLTVLHQDWLNGKEYKCKVSNKALPAPIEKTISKAKGQPREPQVYTLPPSREEMTKNQVSLTCLVKGFYPSDIAVEWESNGQPENNYKTTPPVLDSDGSFFLYSKLTVDKSRWQQGNVFSCSVMHEALHNHYTQKSLSLSPGK

SEQ ID NO: 122 - protein, 350 aa, Artificial Sequence
  MHPD1-A Fc
QVQLVESGGGSVQVGGSLTLSCAASGSDPSIYAMGWFRQAPGKEHEFVAGIGWSAATTYYADSVKGRFGISRDNTKNTVALLMNSLKPEDTAIYYCAADLDHSGFDYWGQGTQVTVSSEPKSCDKTHTCPPCPAPELLGGPSVFLFPPKPKDTLMISRTPEVTCVVVDVSHEDPEVKFNWYVDGVEVHNAKTKPREEQYNSTYRVVSVLTVLHQDWLNGKEYKCKVSNKALPAPIEKTISKAKGQPREPQVYTLPPSREEMTKNQVSLTCLVKGFYPSDIAVEWESNGQPENNYKTTPPVLDSDGSFFLYSKLTVDKSRWQQGNVFSCSVMHEALHNHYTQKSLSLSPGK

SEQ ID NO: 123 - protein, 232 aa, Artificial Sequence
  Fc domain (hIgG1 Fc)
EPKSCDKTHTCPPCPAPELLGGPSVFLFPPKPKDTLMISRTPEVTCVVVDVSHEDPEVKFNWYVDGVEVHNAKTKPREEQYNSTYRVVSVLTVLHQDWLNGKEYKCKVSNKALPAPIEKTISKAKGQPREPQVYTLPPSRDELTKNQVSLTCLVKGFYPSDIAVEWESNGQPENNYKTTPPVLDSDGSFFLYSKLTVDKSRWQQGNVFSCSVMHEALHNHYTQKSLSLSPGK

SEQ ID NO: 124 - protein, 232 aa, Artificial Sequence
  Fc doamin (hIgG1 Fc N297Q)
EPKSCDKTHTCPPCPAPELLGGPSVFLFPPKPKDTLMISRTPEVTCVVVDVSHEDPEVKFNWYVDGVEVHNAKTKPREEQYQSTYRVVSVLTVLHQDWLNGKEYKCKVSNKALPAPIEKTISKAKGQPREPQVYTLPPSRDELTKNQVSLTCLVKGFYPSDIAVEWESNGQPENNYKTTPPVLDSDGSFFLYSKLTVDKSRWQQGNVFSCSVMHEALHNHYTQKSLSLSPGK

SEQ ID NO: 125 - protein, 229 aa, Artificial Sequence
  Fc doamin (hIgG4 Fc S228P)
ESKYGPPCPPCPAPEFLGGPSVFLFPPKPKDTLMISRTPEVTCVVVDVSQEDPEVQFNWYVDGVEVHNAKTKPREEQFNSTYRVVSVLTVLHQDWLNGKEYKCKVSNKGLPSSIEKTISKAKGQPREPQVYTLPPSQEEMTKNQVSLTCLVKGFYPSDIAVEWESNGQPENNYKTTPPVLDSDGSFFLYSRLTVDKSRWQEGNVFSCSVMHEALHNHYTQKSLSLSLGK

SEQ ID NO: 126 - protein, 5 aa, Artificial Sequence
  Keytruda HCDR1
NYYMY

SEQ ID NO: 127 - protein, 17 aa, Artificial Sequence
  Keytruda HCDR2
GINPSNGGTNFNEKFKN

SEQ ID NO: 128 - protein, 11 aa, Artificial Sequence
  Keytruda HCDR3
RDYRFDMGFDY

SEQ ID NO: 129 - protein, 15 aa, Artificial Sequence
  Keytruda LCDR1
RASKGVSTSGYSYLH

SEQ ID NO: 130 - protein, 7 aa, Artificial Sequence
  Keytruda LCDR2
LASYLES

SEQ ID NO: 131 - protein, 9 aa, Artificial Sequence
  Keytruda LCDR3
QHSRDLPLT

SEQ ID NO: 132 - protein, 120 aa, Artificial Sequence [sequence omitted]

SEQ ID NO: 133 - protein, 111 aa, Artificial Sequence [sequence omitted]

SEQ ID NO: 134 - protein, 447 aa, Artificial Sequence
  Keytruda heavy chain
QVQLVQSGVEVKKPGASVKVSCKASGYTFTNYYMYWVRQAPGQGLEWMGGINPSNGGTNFNEKFKNRVTLTTDSSTTTAYMELKSLQFDDTAVYYCARRDYRFDMGFDYWGQGTTVTVSSASTKGPSVFPLAPCSRSTSESTAALGCLVKDYFPEPVTVSWNSGALTSGVHTFPAVLQSSGLYSLSSVVTVPSSSLGTKTYTCNVDHKPSNTKVDKRVESKYGPPCPPCPAPEFLGGPSVFLFPPKPKDTLMISRTPEVTCVVVDVSQEDPEVQFNWYVDGVEVHNAKTKPREEQFNSTYRVVSVLTVLHQDWLNGKEYKCKVSNKGLPSSIEKTISKAKGQPREPQVYTLPPSQEEMTKNQVSLTCLVKGFYPSDIAVEWESNGQPENNYKTTPPVLDSDGSFFLYSRLTVDKSRWQEGNVFSCSVMHEALHNHYTQKSLSLSLGK

SEQ ID NO: 135 - protein, 218 aa, Artificial Sequence
  Keytruda light chain
EIVLTQSPATLSLSPGERATLSCRASKGVSTSGYSYLHWYQQKPGQAPRLLIYLASYLESGVPARFSGSGSGTDFTLTISSLEPEDFAVYYCQHSRDLPLTFGGGTKVEIKRTVAAPSVFIFPPSDEQLKSGTASVVCLLNNFYPREAKVQWKVDNALQSGNSQESVTEQDSKDSTYSLSSTLTLSKADYEKHKVYACEVTHQGLSSPVTKSFNRGEC

SEQ ID NO: 136 - protein, 8 aa, Artificial Sequence
  HCDR1 general formula 1
  misc_feature (1)..(1): Xaa = Ala, Gly, His, Lys, Ser or Val
  misc_feature (2)..(2): Xaa = Ala, Gly, His, Leu, Asn, Pro, Arg, Ser, Thr or Val
  misc_feature (3)..(3): Xaa = Asp, Glu, Phe, Gly, Ile, Lys, Gln, Arg, Ser or Val
  misc_feature (4)..(4): Xaa = Asp, Gly, His, Lys, Leu, Pro, Gln, Arg, Ser, Thr, Val or Tyr
  misc_feature (5)..(5): Xaa = Ala, Phe, Asn, Gln, Arg, Ser or Thr
XXXXXIYA

SEQ ID NO: 137 - protein, 8 aa, Artificial Sequence
  HCDR2 general formula 1
  misc_feature (1)..(1): Xaa = Ile or Leu
  misc_feature (4)..(4): Xaa = Ala, Asn, Arg or Ser
  misc_feature (5)..(5): Xaa = Ala, Phe, Trp or Tyr
  misc_feature (6)..(6): Xaa = Ala, Gly or Ser
  misc_feature (8)..(8): Xaa = Glu, Gln, Ser or Thr
XGWXXXTX

SEQ ID NO: 138 - protein, 11 aa, Artificial Sequence
  HCDR3 general formula 1
  misc_feature (4)..(4): Xaa = Ile or Leu
  misc_feature (6)..(6): Xaa = His, Arg or Val
  misc_feature (7)..(7): Xaa = Ala, Asp, Gly, His, Leu, Asn, Arg, Ser, Thr or Val
AADXDXXGFDY

SEQ ID NO: 139 - protein, 118 aa, Artificial Sequence
  VHH general formula 1
  misc_feature (26)..(26): Xaa = Ala, Gly, His, Lys, Ser or Val
  misc_feature (27)..(27): Xaa = Ala, Gly, His, Leu, Asn, Pro, Arg, Ser, Thr or Val
  misc_feature (28)..(28): Xaa = Asp, Glu, Phe, Gly, Ile, Lys, Gln, Arg, Ser or Val
  misc_feature (29)..(29): Xaa = Asp, Gly, His, Lys, Leu, Pro, Gln, Arg, Ser, Thr, Val or Tyr
  misc_feature (30)..(30): Xaa = Ala, Phe, Asn, Gln, Arg, Ser or Thr
  misc_feature (51)..(51): Xaa = Ile or Leu
  misc_feature (54)..(54): Xaa = Ala, Asn, Arg or Ser
  misc_feature (55)..(55): Xaa = Ala, Phe, Trp or Tyr
  misc_feature (56)..(56): Xaa = Ala, Gly or Ser
  misc_feature (58)..(58): Xaa = Glu, Gln, Ser or Thr
  misc_feature (100)..(100): Xaa = Ile or Leu
  misc_feature (102)..(102): Xaa = His, Arg or Val
  misc_feature (103)..(103): Xaa = Ala, Asp, Gly, His, Leu, Asn, Arg, Ser, Thr or Val
QVQLVESGGGSVQVGGSLTLSCAASXXXXXIYAMGWFRQAPGKEHEFVAGXGWXXXTXYYADSVKGRFGISRDNTKNTVALLMNSLKPEDTAIYYCAADXDXXGFDYWGQGTQVTVSS

SEQ ID NO: 140 - protein, 8 aa, Artificial Sequence
  HCDR1 general formula 2
  misc_feature (1)..(1): Xaa = Gly, His or Lys
  misc_feature (2)..(2): Xaa = Ala, Gly, Leu, Asn, Ser or Val
  misc_feature (3)..(3): Xaa = Asp, Arg or Val
  misc_feature (4)..(4): Xaa = Gly, His, Pro, Gln, Arg or Thr
  misc_feature (5)..(5): Xaa = Arg, Ser or Thr
XXXXXIYA

SEQ ID NO: 141 - protein, 8 aa, Artificial Sequence
  HCDR2 general formula 2
  misc_feature (4)..(4): Xaa = Ala or Asn
  misc_feature (5)..(5): Xaa = Phe or Tyr
  misc_feature (6)..(6): Xaa = Ala or Ser
  misc_feature (8)..(8): Xaa = Glu, Gln or Thr
IGWXXXTX

SEQ ID NO: 142 - protein, 11 aa, Artificial Sequence
  HCDR3 general formula 2
  misc_feature (4)..(4): Xaa = Ile or Leu
  misc_feature (6)..(6): Xaa = His or Arg
  misc_feature (7)..(7): Xaa = Ala, His or Ser
AADXDXXGFDY

SEQ ID NO: 143 - protein, 118 aa, Artificial Sequence
  VHH general formula 2
  misc_feature (26)..(26): Xaa = Gly, His or Lys
  misc_feature (27)..(27): Xaa = Ala, Gly, Leu, Asn, Ser or Val
  misc_feature (28)..(28): Xaa = Asp, Arg or Val
  misc_feature (29)..(29): Xaa = Gly, His, Pro, Gln, Arg or Thr
  misc_feature (30)..(30): Xaa = Arg, Ser or Thr
  misc_feature (54)..(54): Xaa = Ala or Asn
  misc_feature (55)..(55): Xaa = Phe or Tyr
  misc_feature (56)..(56): Xaa = Ala or Ser
  misc_feature (58)..(58): Xaa = Glu, Gln or Thr
  misc_feature (100)..(100): Xaa = Ile or Leu
  misc_feature (102)..(102): Xaa = His or Arg
  misc_feature (103)..(103): Xaa = Ala, His or Ser
QVQLVESGGGSVQVGGSLTLSCAASXXXXXIYAMGWFRQAPGKEHEFVAGIGWXXXTXYYADSVKGRFGISRDNTKNTVALLMNSLKPEDTAIYYCAADXDXXGFDYWGQGTQVTVSS

SEQ ID NO: 144 - protein, 25 aa, Artificial Sequence
  MHPD1-A-H1 H-FR1
QVQLVESGGGSVQPGGSLTLSCAAS

SEQ ID NO: 145 - protein, 25 aa, Artificial Sequence
  MHPD1-A-H2 H-FR1
QVQLVESGGGSVQVGGSLRLSCAAS

SEQ ID NO: 146 - protein, 25 aa, Artificial Sequence
  MHPD1-A-H9-10+12+14-15+17 H-FR1
QVQLVESGGGSVQPGGSLRLSCAAS

SEQ ID NO: 147 - protein, 25 aa, Artificial Sequence
  MHPD1-A-1-6+8-14+H16+18-19 H-FR1
QVQLVESGGGLVQPGGSLRLSCAAS

SEQ ID NO: 148 - protein, 25 aa, Artificial Sequence
  MHPD1-A-7+15-49 H-FR1
QVQLVESGGGLVQPGGSLRLSCATS

SEQ ID NO: 149 - protein, 17 aa, Artificial Sequence
  MHPD1-A-H6-7 H-FR2
MMWFRQAPGKEHEFVAG

SEQ ID NO: 150 - protein, 17 aa, Artificial Sequence
  MHPD1-A-1-49 H8+17-19 H-FR2
MGWFRQAPGKGLEFVAG

SEQ ID NO: 151 - protein, 17 aa, Artificial Sequence
  MHPD1-A-34 H-FR2
AGWFRQAPGKGLEFVAG

SEQ ID NO: 152 - protein, 38 aa, Artificial Sequence
  MHPD1-A-H2+9 H-FR3
YYADSVKGRFGISRDNTKNTVALLMNSLRAEDTAIYYC

SEQ ID NO: 153 - protein, 38 aa, Artificial Sequence
  MHPD1-A-H3 H-FR3
YYADSVKGRFGISRDNTKNTLALLMNSLKPEDTAIYYC

SEQ ID NO: 154 - protein, 38 aa, Artificial Sequence
  MHPD1-A-H5 H-FR3
YYADSVKGRFGISRDNTKNTVYLQMNSLKPEDTAIYYC

SEQ ID NO: 155 - protein, 38 aa, Artificial Sequence
  MHPD1-A-H7 H-FR3
YYADSVKGRFGISRDNSKNTVALLMNSLKPEDTAIYYC

SEQ ID NO: 156 - protein, 38 aa, Artificial Sequence
  MHPD1-A-H10 H-FR3
YYADSVKGRFTISRDNTKNTLALLMNSLKPEDTAIYYC

SEQ ID NO: 157 - protein, 38 aa, Artificial Sequence
  MHPD1-A-H12 H-FR3
YYADSVKGRFTISRDNTKNTLALLMNSLRAEDTAIYYC

SEQ ID NO: 158 - protein, 38 aa, Artificial Sequence
  MHPD1-A-H14 H-FR3
YYADSVKGRFGISRDNTKNTVYLQMNSLRAEDTAIYYC

SEQ ID NO: 159 - protein, 38 aa, Artificial Sequence
  MHPD1-A-H15+17-18 H-FR3
YYADSVKGRFTISRDNTKNTLYLQMNSLRAEDTAIYYC

SEQ ID NO: 160 - protein, 38 aa, Artificial Sequence
  MHPD1-A-H16 H-FR3
YYADSVKGRFGISRDNTKNTVALLMNSLRAEDTAVYYC

SEQ ID NO: 161 - protein, 38 aa, Artificial Sequence
  MHPD1-A-1-49+H19 H-FR3
YYADSVKGRFTISRDNTKNTLYLQMNSLRAEDTAVYYC

SEQ ID NO: 162 - protein, 11 aa, Artificial Sequence
  MHPD1-A-1-49+H1+9-10+12+14-19 H-FR4
WGQGTLVTVSS

SEQ ID NO: 163 - protein, 118 aa, Artificial Sequence
  MHPD1-A-H1
QVQLVESGGGSVQPGGSLTLSCAASGSDPSIYAMGWFRQAPGKEHEFVAGIGWSAATTYYADSVKGRFGISRDNTKNTVALLMNSLKPEDTAIYYCAADLDHSGFDYWGQGTLVTVSS

SEQ ID NO: 164 - protein, 118 aa, Artificial Sequence
  MHPD1-A-H2
QVQLVESGGGSVQVGGSLRLSCAASGSDPSIYAMGWFRQAPGKEHEFVAGIGWSAATTYYADSVKGRFGISRDNTKNTVALLMNSLRAEDTAIYYCAADLDHSGFDYWGQGTQVTVSS

SEQ ID NO: 165 - protein, 118 aa, Artificial Sequence
  MHPD1-A-H3
QVQLVESGGGSVQVGGSLTLSCAASGSDPSIYAMGWFRQAPGKEHEFVAGIGWSAATTYYADSVKGRFGISRDNTKNTLALLMNSLKPEDTAIYYCAADLDHSGFDYWGQGTQVTVSS

SEQ ID NO: 166 - protein, 118 aa, Artificial Sequence
  MHPD1-A-H5
QVQLVESGGGSVQVGGSLTLSCAASGSDPSIYAMGWFRQAPGKEHEFVAGIGWSAATTYYADSVKGRFGISRDNTKNTVYLQMNSLKPEDTAIYYCAADLDHSGFDYWGQGTQVTVSS

SEQ ID NO: 167 - protein, 118 aa, Artificial Sequence
  MHPD1-A-H6
QVQLVESGGGSVQVGGSLTLSCAASGSDPSIYAMMWFRQAPGKEHEFVAGIGWSAATTYYADSVKGRFGISRDNTKNTVALLMNSLKPEDTAIYYCAADLDHSGFDYWGQGTQVTVSS

SEQ ID NO: 168 - protein, 118 aa, Artificial Sequence
  MHPD1-A-H7
QVQLVESGGGSVQVGGSLTLSCAASGSDPSIYAMMWFRQAPGKEHEFVAGIGWSAATTYYADSVKGRFGISRDNSKNTVALLMNSLKPEDTAIYYCAADLDHSGFDYWGQGTQVTVSS

SEQ ID NO: 169 - protein, 118 aa, Artificial Sequence
  MHPD1-A-H8
QVQLVESGGGSVQVGGSLTLSCAASGSDPSIYAMGWFRQAPGKGLEFVAGIGWSAATTYYADSVKGRFGISRDNTKNTVALLMNSLKPEDTAIYYCAADLDHSGFDYWGQGTQVTVSS

SEQ ID NO: 170 - protein, 118 aa, Artificial Sequence
  MHPD1-A-H9
QVQLVESGGGSVQPGGSLRLSCAASGSDPSIYAMGWFRQAPGKEHEFVAGIGWSAATTYYADSVKGRFGISRDNTKNTVALLMNSLRAEDTAIYYCAADLDHSGFDYWGQGTLVTVSS

SEQ ID NO: 171 - protein, 118 aa, Artificial Sequence
  MHPD1-A-H10
QVQLVESGGGSVQPGGSLRLSCAASGSDPSIYAMGWFRQAPGKEHEFVAGIGWSAATTYYADSVKGRFTISRDNTKNTLALLMNSLKPEDTAIYYCAADLDHSGFDYWGQGTLVTVSS

SEQ ID NO: 172 - protein, 118 aa, Artificial Sequence
  MHPD1-A-H12
QVQLVESGGGSVQPGGSLRLSCAASGSDPSIYAMGWFRQAPGKEHEFVAGIGWSAATTYYADSVKGRFTISRDNTKNTLALLMNSLRAEDTAIYYCAADLDHSGFDYWGQGTLVTVSS

SEQ ID NO: 173 - protein, 118 aa, Artificial Sequence
  MHPD1-A-H14
QVQLVESGGGSVQPGGSLRLSCAASGSDPSIYAMGWFRQAPGKEHEFVAGIGWSAATTYYADSVKGRFGISRDNTKNTVYLQMNSLRAEDTAIYYCAADLDHSGFDYWGQGTLVTVSS

SEQ ID NO: 174 - protein, 118 aa, Artificial Sequence
  MHPD1-A-H15
QVQLVESGGGSVQPGGSLRLSCAASGSDPSIYAMGWFRQAPGKEHEFVAGIGWSAATTYYADSVKGRFTISRDNTKNTLYLQMNSLRAEDTAIYYCAADLDHSGFDYWGQGTLVTVSS

SEQ ID NO: 175 - protein, 118 aa, Artificial Sequence
  MHPD1-A-H16
QVQLVESGGGLVQPGGSLRLSCAASGSDPSIYAMGWFRQAPGKEHEFVAGIGWSAATTYYADSVKGRFGISRDNTKNTVALLMNSLRAEDTAVYYCAADLDHSGFDYWGQGTLVTVSS

SEQ ID NO: 176 - protein, 118 aa, Artificial Sequence
  MHPD1-A-H17
QVQLVESGGGSVQPGGSLRLSCAASGSDPSIYAMGWFRQAPGKGLEFVAGIGWSAATTYYADSVKGRFTISRDNTKNTLYLQMNSLRAEDTAIYYCAADLDHSGFDYWGQGTLVTVSS

SEQ ID NO: 177 - protein, 118 aa, Artificial Sequence
  MHPD1-A-H18
QVQLVESGGGLVQPGGSLRLSCAASGSDPSIYAMGWFRQAPGKGLEFVAGIGWSAATTYYADSVKGRFTISRDNTKNTLYLQMNSLRAEDTAIYYCAADLDHSGFDYWGQGTLVTVSS

SEQ ID NO: 178 - protein, 118 aa, Artificial Sequence
  MHPD1-A-H19
QVQLVESGGGLVQPGGSLRLSCAASGSDPSIYAMGWFRQAPGKGLEFVAGIGWSAATTYYADSVKGRFTISRDNTKNTLYLQMNSLRAEDTAVYYCAADLDHSGFDYWGQGTLVTVSS

SEQ ID NO: 179 - protein, 118 aa, Artificial Sequence
  MHPD1-A-1 H
QVQLVESGGGLVQPGGSLRLSCAASGSDPSIYAMGWFRQAPGKGLEFVAGIGWAWATTYYADSVKGRFTISRDNTKNTLYLQMNSLRAEDTAVYYCAADLDRSGFDYWGQGTLVTVSS

SEQ ID NO: 180 - protein, 118 aa, Artificial Sequence
  MHPD1-A-2 H
QVQLVESGGGLVQPGGSLRLSCAASGRFPSIYAMGWFRQAPGKGLEFVAGIGWRYATTYYADSVKGRFTISRDNTKNTLYLQMNSLRAEDTAVYYCAADLDHSGFDYWGQGTLVTVSS

SEQ ID NO: 181 - protein, 118 aa, Artificial Sequence
  MHPD1-A-3 H
QVQLVESGGGLVQPGGSLRLSCAASGSGRSIYAMGWFRQAPGKGLEFVAGIGWSYATTYYADSVKGRFTISRDNTKNTLYLQMNSLRAEDTAVYYCAADLDHSGFDYWGQGTLVTVSS

SEQ ID NO: 182 - protein, 118 aa, Artificial Sequence
  MHPD1-A-4 H
QVQLVESGGGLVQPGGSLRLSCAASGSVGSIYAMGWFRQAPGKGLEFVAGIGWAFATTYYADSVKGRFTISRDNTKNTLYLQMNSLRAEDTAVYYCAADLDHSGFDYWGQGTLVTVSS

SEQ ID NO: 183 - protein, 118 aa, Artificial Sequence
  MHPD1-A-5 H
QVQLVESGGGLVQPGGSLRLSCAASGSSLSIYAMGWFRQAPGKGLEFVAGIGWAYATTYYADSVKGRFTISRDNTKNTLYLQMNSLRAEDTAVYYCAADLDHSGFDYWGQGTLVTVSS

SEQ ID NO: 184 - protein, 118 aa, Artificial Sequence
  MHPD1-A-6 H
QVQLVESGGGLVQPGGSLRLSCAASGRRPSIYAMGWFRQAPGKGLEFVAGIGWNYATTYYADSVKGRFTISRDNTKNTLYLQMNSLRAEDTAVYYCAADLDHSGFDYWGQGTLVTVSS

SEQ ID NO: 185 - protein, 118 aa, Artificial Sequence
  MHPD1-A-7 H
QVQLVESGGGLVQPGGSLRLSCATSGSRRSIYAMGWFRQAPGKGLEFVAGIGWAYATTYYADSVKGRFTISRDNTKNTLYLQMNSLRAEDTAVYYCAADLDHSGFDYWGQGTLVTVSS

SEQ ID NO: 186 - protein, 118 aa, Artificial Sequence
  MHPD1-A-8 H
QVQLVESGGGLVQPGGSLRLSCAASGGRPSIYAMGWFRQAPGKGLEFVAGIGWAFATTYYADSVKGRFTISRDNTKNTLYLQMNSLRAEDTAVYYCAADLDHSGFDYWGQGTLVTVSS

SEQ ID NO: 187 - protein, 118 aa, Artificial Sequence
  MHPD1-A-9 H
QVQLVESGGGLVQPGGSLRLSCAASGSGHSIYAMGWFRQAPGKGLEFVAGIGWSYATTYYADSVKGRFTISRDNTKNTLYLQMNSLRAEDTAVYYCAADLDHSGFDYWGQGTLVTVSS

SEQ ID NO: 188 - protein, 118 aa, Artificial Sequence
  MHPD1-A-10 H
QVQLVESGGGLVQPGGSLRLSCAASGSDDRIYAMGWFRQAPGKGLEFVAGIGWRYATTYYADSVKGRFTISRDNTKNTLYLQMNSLRAEDTAVYYCAADLDHSGFDYWGQGTLVTVSS

SEQ ID NO: 189 - protein, 118 aa, Artificial Sequence
  MHPD1-A-11 H
QVQLVESGGGLVQPGGSLRLSCAASGSQLSIYAMGWFRQAPGKGLEFVAGIGWRFATTYYADSVKGRFTISRDNTKNTLYLQMNSLRAEDTAVYYCAADLDHSGFDYWGQGTLVTVSS

SEQ ID NO: 190 - protein, 118 aa, Artificial Sequence
  MHPD1-A-12 H
QVQLVESGGGLVQPGGSLRLSCAASGSDYAIYAMGWFRQAPGKGLEFVAGIGWAFATTYYADSVKGRFTISRDNTKNTLYLQMNSLRAEDTAVYYCAADLDHSGFDYWGQGTLVTVSS

SEQ ID NO: 191 - protein, 118 aa, Artificial Sequence
  MHPD1-A-13 H
QVQLVESGGGLVQPGGSLRLSCAASHADPSIYAMGWFRQAPGKGLEFVAGIGWNYATTYYADSVKGRFTISRDNTKNTLYLQMNSLRAEDTAVYYCAADLDHSGFDYWGQGTLVTVSS

SEQ ID NO: 192 - protein, 118 aa, Artificial Sequence
  MHPD1-A-14 H
QVQLVESGGGLVQPGGSLRLSCAASSHRPSIYAMGWFRQAPGKGLEFVAGIGWRYATTYYADSVKGRFTISRDNTKNTLYLQMNSLRAEDTAVYYCAADLDHSGFDYWGQGTLVTVSS

SEQ ID NO: 193 - protein, 118 aa, Artificial Sequence
  MHPD1-A-15 H
QVQLVESGGGLVQPGGSLRLSCATSGLRRSIYAMGWFRQAPGKGLEFVAGIGWAYSTTYYADSVKGRFTISRDNTKNTLYLQMNSLRAEDTAVYYCAADLDHSGFDYWGQGTLVTVSS

SEQ ID NO: 194 - protein, 118 aa, Artificial Sequence
  MHPD1-A-16 H
QVQLVESGGGLVQPGGSLRLSCATSGSRVSIYAMGWFRQAPGKGLEFVAGIGWAYATTYYADSVKGRFTISRDNTKNTLYLQMNSLRAEDTAVYYCAADLDHSGFDYWGQGTLVTVSS

SEQ ID NO: 195 - protein, 118 aa, Artificial Sequence
  MHPD1-A-17 H
QVQLVESGGGLVQPGGSLRLSCATSGSISSIYAMGWFRQAPGKGLEFVAGIGWAYATTYYADSVKGRFTISRDNTKNTLYLQMNSLRAEDTAVYYCAADLDHSGFDYWGQGTLVTVSS

SEQ ID NO: 196 - protein, 118 aa, Artificial Sequence
  MHPD1-A-18 H
QVQLVESGGGLVQPGGSLRLSCATSGSRSSIYAMGWFRQAPGKGLEFVAGLGWAYATTYYADSVKGRFTISRDNTKNTLYLQMNSLRAEDTAVYYCAADLDHLGFDYWGQGTLVTVSS

SEQ ID NO: 197 - protein, 118 aa, Artificial Sequence
  MHPD1-A-19 H
QVQLVESGGGLVQPGGSLRLSCATSGSEVSIYAMGWFRQAPGKGLEFVAGIGWAYATTYYADSVKGRFTISRDNTKNTLYLQMNSLRAEDTAVYYCAADLDRRGFDYWGQGTLVTVSS

SEQ ID NO: 198 - protein, 118 aa, Artificial Sequence
  MHPD1-A-20 H
QVQLVESGGGLVQPGGSLRLSCATSGSRKSIYAMGWFRQAPGKGLEFVAGIGWAYATTYYADSVKGRFTISRDNTKNTLYLQMNSLRAEDTAVYYCAADLDHSGFDYWGQGTLVTVSS

SEQ ID NO: 199 - protein, 118 aa, Artificial Sequence
  MHPD1-A-21 H
QVQLVESGGGLVQPGGSLRLSCATSGSRRSIYAMGWFRQAPGKGLEFVAGIGWAYATSYYADSVKGRFTISRDNTKNTLYLQMNSLRAEDTAVYYCAADLDHSGFDYWGQGTLVTVSS

SEQ ID NO: 200 - protein, 118 aa, Artificial Sequence
  MHPD1-A-22 H
QVQLVESGGGLVQPGGSLRLSCATSGSRRSIYAMGWFRQAPGKGLEFVAGIGWAYATTYYADSVKGRFTISRDNTKNTLYLQMNSLRAEDTAVYYCAADLDRGGFDYWGQGTLVTVSS

SEQ ID NO: 201 - protein, 118 aa, Artificial Sequence
  MHPD1-A-23 H
QVQLVESGGGLVQPGGSLRLSCATSGTRRSIYAMGWFRQAPGKGLEFVAGIGWAYATTYYADSVKGRFTISRDNTKNTLYLQMNSLRAEDTAVYYCAADLDHSGFDYWGQGTLVTVSS

SEQ ID NO: 202 - protein, 118 aa, Artificial Sequence
  MHPD1-A-24 H
QVQLVESGGGLVQPGGSLRLSCATSGSRHSIYAMGWFRQAPGKGLEFVAGIGWAYATTYYADSVKGRFTISRDNTKNTLYLQMNSLRAEDTAVYYCAADLDRAGFDYWGQGTLVTVSS

SEQ ID NO: 203 - protein, 118 aa, Artificial Sequence
  MHPD1-A-25 H
QVQLVESGGGLVQPGGSLRLSCATSGVRRSIYAMGWFRQAPGKGLEFVAGIGWAYATTYYADSVKGRFTISRDNTKNTLYLQMNSLRAEDTAVYYCAADLDRHGFDYWGQGTLVTVSS

SEQ ID NO: 204 - protein, 118 aa, Artificial Sequence
  MHPD1-A-26 H
QVQLVESGGGLVQPGGSLRLSCATSGSRSNIYAMGWFRQAPGKGLEFVAGIGWAYATTYYADSVKGRFTISRDNTKNTLYLQMNSLRAEDTAVYYCAADLDRDGFDYWGQGTLVTVSS

SEQ ID NO: 205 - protein, 118 aa, Artificial Sequence
  MHPD1-A-27 H
QVQLVESGGGLVQPGGSLRLSCATSKSRRSIYAMGWFRQAPGKGLEFVAGIGWAYATTYYADSVKGRFTISRDNTKNTLYLQMNSLRAEDTAVYYCAADLDHSGFDYWGQGTLVTVSS

SEQ ID NO: 206 - protein, 118 aa, Artificial Sequence
  MHPD1-A-28 H
QVQLVESGGGLVQPGGSLRLSCATSKLRRSIYAMGWFRQAPGKGLEFVAGIGWAYATQYYADSVKGRFTISRDNTKNTLYLQMNSLRAEDTAVYYCAADLDHSGFDYWGQGTLVTVSS

SEQ ID NO: 207 - protein, 118 aa, Artificial Sequence
  MHPD1-A-29 H
QVQLVESGGGLVQPGGSLRLSCATSGSGGSIYAMGWFRQAPGKGLEFVAGIGWAYATTYYADSVKGRFTISRDNTKNTLYLQMNSLRAEDTAVYYCAADLDHSGFDYWGQGTLVTVSS

SEQ ID NO: 208 - protein, 118 aa, Artificial Sequence
  MHPD1-A-30 H
QVQLVESGGGLVQPGGSLRLSCATSGVRRSIYAMGWFRQAPGKGLEFVAGIGWAYATQYYADSVKGRFTISRDNTKNTLYLQMNSLRAEDTAVYYCAADIDHSGFDYWGQGTLVTVSS

SEQ ID NO: 209 - protein, 118 aa, Artificial Sequence
  MHPD1-A-31 H
QVQLVESGGGLVQPGGSLRLSCATSGSRRSIYAMGWFRQAPGKGLEFVAGLGWAYATTYYADSVKGRFTISRDNTKNTLYLQMNSLRAEDTAVYYCAADLDHHGFDYWGQGTLVTVSS

SEQ ID NO: 210 - protein, 118 aa, Artificial Sequence
  MHPD1-A-32 H
QVQLVESGGGLVQPGGSLRLSCATSKNRRSIYAMGWFRQAPGKGLEFVAGIGWAYATTYYADSVKGRFTISRDNTKNTLYLQMNSLRAEDTAVYYCAADLDHSGFDYWGQGTLVTVSS

SEQ ID NO: 211 - protein, 118 aa, Artificial Sequence
  MHPD1-A-33 H
QVQLVESGGGLVQPGGSLRLSCATSGSRSQIYAMGWFRQAPGKGLEFVAGIGWAYATTYYADSVKGRFTISRDNTKNTLYLQMNSLRAEDTAVYYCAADLDHSGFDYWGQGTLVTVSS

SEQ ID NO: 212 - protein, 118 aa, Artificial Sequence
  MHPD1-A-34 H
QVQLVESGGGLVQPGGSLRLSCATSGSRRSIYAAGWFRQAPGKGLEFVAGIGWAYATTYYADSVKGRFTISRDNTKNTLYLQMNSLRAEDTAVYYCAADLDHSGFDYWGQGTLVTVSS

SEQ ID NO: 213 - protein, 118 aa, Artificial Sequence
  MHPD1-A-35 H
QVQLVESGGGLVQPGGSLRLSCATSAPRRSIYAMGWFRQAPGKGLEFVAGIGWAYGTTYYADSVKGRFTISRDNTKNTLYLQMNSLRAEDTAVYYCAADLDHSGFDYWGQGTLVTVSS

SEQ ID NO: 214 - protein, 118 aa, Artificial Sequence
  MHPD1-A-36 H
QVQLVESGGGLVQPGGSLRLSCATSGSRRFIYAMGWFRQAPGKGLEFVAGIGWAYATQYYADSVKGRFTISRDNTKNTLYLQMNSLRAEDTAVYYCAADLDHSGFDYWGQGTLVTVSS

SEQ ID NO: 215 - protein, 118 aa, Artificial Sequence
  MHPD1-A-37 H
QVQLVESGGGLVQPGGSLRLSCATSGARRSIYAMGWFRQAPGKGLEFVAGIGWAYATTYYADSVKGRFTISRDNTKNTLYLQMNSLRAEDTAVYYCAADLDRTGFDYWGQGTLVTVSS

SEQ ID NO: 216 - protein, 118 aa, Artificial Sequence
  MHPD1-A-38 H
QVQLVESGGGLVQPGGSLRLSCATSGNRRSIYAMGWFRQAPGKGLEFVAGIGWAYATTYYADSVKGRFTISRDNTKNTLYLQMNSLRAEDTAVYYCAADLDRRGFDYWGQGTLVTVSS

SEQ ID NO: 217 - protein, 118 aa, Artificial Sequence
  MHPD1-A-39 H
QVQLVESGGGLVQPGGSLRLSCATSGSRRSIYAMGWFRQAPGKGLEFVAGIGWAYATEYYADSVKGRFTISRDNTKNTLYLQMNSLRAEDTAVYYCAADLDHSGFDYWGQGTLVTVSS

SEQ ID NO: 218 - protein, 118 aa, Artificial Sequence
  MHPD1-A-40 H
QVQLVESGGGLVQPGGSLRLSCATSGSRRSIYAMGWFRQAPGKGLEFVAGIGWAYATTYYADSVKGRFTISRDNTKNTLYLQMNSLRAEDTAVYYCAADLDVAGFDYWGQGTLVTVSS

SEQ ID NO: 219 - protein, 118 aa, Artificial Sequence
  MHPD1-A-41 H
QVQLVESGGGLVQPGGSLRLSCATSVSRRSIYAMGWFRQAPGKGLEFVAGIGWAYATTYYADSVKGRFTISRDNTKNTLYLQMNSLRAEDTAVYYCAADLDHSGFDYWGQGTLVTVSS

SEQ ID NO: 220 - protein, 118 aa, Artificial Sequence
  MHPD1-A-42 H
QVQLVESGGGLVQPGGSLRLSCATSGSRQTIYAMGWFRQAPGKGLEFVAGIGWAYATQYYADSVKGRFTISRDNTKNTLYLQMNSLRAEDTAVYYCAADLDHSGFDYWGQGTLVTVSS

SEQ ID NO: 221 - protein, 118 aa, Artificial Sequence
  MHPD1-A-43 H
QVQLVESGGGLVQPGGSLRLSCATSGSRRSIYAMGWFRQAPGKGLEFVAGIGWAYATTYYADSVKGRFTISRDNTKNTLYLQMNSLRAEDTAVYYCAADLDRAGFDYWGQGTLVTVSS

SEQ ID NO: 222 - protein, 118 aa, Artificial Sequence
  MHPD1-A-44 H
QVQLVESGGGLVQPGGSLRLSCATSGSRTRIYAMGWFRQAPGKGLEFVAGIGWAYATEYYADSVKGRFTISRDNTKNTLYLQMNSLRAEDTAVYYCAADLDHSGFDYWGQGTLVTVSS

SEQ ID NO: 223 - protein, 118 aa, Artificial Sequence
  MHPD1-A-45 H
QVQLVESGGGLVQPGGSLRLSCATSHLRRSIYAMGWFRQAPGKGLEFVAGIGWAYATTYYADSVKGRFTISRDNTKNTLYLQMNSLRAEDTAVYYCAADLDHSGFDYWGQGTLVTVSS

SEQ ID NO: 224 - protein, 118 aa, Artificial Sequence
  MHPD1-A-46 H
QVQLVESGGGLVQPGGSLRLSCATSGSKGSIYAMGWFRQAPGKGLEFVAGIGWAYATTYYADSVKGRFTISRDNTKNTLYLQMNSLRAEDTAVYYCAADLDRSGFDYWGQGTLVTVSS

SEQ ID NO: 225 - protein, 118 aa, Artificial Sequence
  MHPD1-A-47 H
QVQLVESGGGLVQPGGSLRLSCATSGSRLSIYAMGWFRQAPGKGLEFVAGIGWAYATTYYADSVKGRFTISRDNTKNTLYLQMNSLRAEDTAVYYCAADLDHSGFDYWGQGTLVTVSS

SEQ ID NO: 226 - protein, 118 aa, Artificial Sequence
  MHPD1-A-48 H
QVQLVESGGGLVQPGGSLRLSCATSGSRRSIYAMGWFRQAPGKGLEFVAGIGWAYATTYYADSVKGRFTISRDNTKNTLYLQMNSLRAEDTAVYYCAADLDRNGFDYWGQGTLVTVSS

SEQ ID NO: 227 - protein, 118 aa, Artificial Sequence
  MHPD1-A-49 H
QVQLVESGGGLVQPGGSLRLSCATSGSRRSIYAMGWFRQAPGKGLEFVAGIGWAYATTYYADSVKGRFTISRDNTKNTLYLQMNSLRAEDTAVYYCAADLDRVGFDYWGQGTLVTVSS

SEQ ID NO: 228 - protein, 232 aa, Artificial Sequence
  Fc domain (hIgG1 Fc C220A L234A L235A)
EPKSADKTHTCPPCPAPEAAGGPSVFLFPPKPKDTLMISRTPEVTCVVVDVSHEDPEVKFNWYVDGVEVHNAKTKPREEQYNSTYRVVSVLTVLHQDWLNGKEYKCKVSNKALPAPIEKTISKAKGQPREPQVYTLPPSREEMTKNQVSLTCLVKGFYPSDIAVEWESNGQPENNYKTTPPVLDSDGSFFLYSKLTVDKSRWQQGNVFSCSVMHEALHNHYTQKSLSLSPGK

SEQ ID NO: 229 - protein, 232 aa, Artificial Sequence
  Fc domain (hIgG1 Fc C220S L234A L235A)
EPKSSDKTHTCPPCPAPEAAGGPSVFLFPPKPKDTLMISRTPEVTCVVVDVSHEDPEVKFNWYVDGVEVHNAKTKPREEQYNSTYRVVSVLTVLHQDWLNGKEYKCKVSNKALPAPIEKTISKAKGQPREPQVYTLPPSREEMTKNQVSLTCLVKGFYPSDIAVEWESNGQPENNYKTTPPVLDSDGSFFLYSKLTVDKSRWQQGNVFSCSVMHEALHNHYTQKSLSLSPGK

SEQ ID NO: 230 - protein, 25 aa, Artificial Sequence
  H-FR1 general formula 1
  misc_feature (11)..(11): Xaa = Leu or Ser
  misc_feature (14)..(14): Xaa = Pro or Val
  misc_feature (19)..(19): Xaa = Arg or Thr
  misc_feature (24)..(24): Xaa = Ala or Thr
QVQLVESGGGXVQXGGSLXLSCAXS

SEQ ID NO: 231 - protein, 17 aa, Artificial Sequence
  H-FR2 general formula 1
  misc_feature (1)..(1): Xaa = Ala or Met
  misc_feature (2)..(2): Xaa = Gly or Met
  misc_feature (11)..(11): Xaa = Glu or Gly
  misc_feature (12)..(12): Xaa = His or Leu
XXWFRQAPGKXXEFVAG

SEQ ID NO: 232 - protein, 38 aa, Artificial Sequence
  H-FR3 general formula 1
  misc_feature (11)..(11): Xaa = Gly or Thr
  misc_feature (17)..(17): Xaa = Ser or Thr
  misc_feature (21)..(21): Xaa = Leu or Val
  misc_feature (22)..(22): Xaa = Ala or Tyr
  misc_feature (24)..(24): Xaa = Leu or Gln
  misc_feature (29)..(29): Xaa = Lys or Arg
  misc_feature (30)..(30): Xaa = Ala or Pro
  misc_feature (35)..(35): Xaa = Ile or Val
YYADSVKGRFXISRDNXKNTXXLXMNSLXXEDTAXYYC

SEQ ID NO: 233 - protein, 11 aa, Artificial Sequence
  H-FR4 general formula 1
  misc_feature (6)..(6): Xaa = Leu or Gln
WGQGTXVTVSS

SEQ ID NO: 234 - protein, 118 aa, Artificial Sequence
  VHH H general formula 1
  misc_feature (11)..(11): Xaa = Leu or Ser
  misc_feature (14)..(14): Xaa = Pro or Val
  misc_feature (19)..(19): Xaa = Arg or Thr
  misc_feature (24)..(24): Xaa = Ala or Thr
  misc_feature (26)..(26): Xaa = Ala, Gly, His, Lys, Ser or Val
  misc_feature (27)..(27): Xaa = Ala, Gly, His, Leu, Asn, Pro, Arg, Ser, Thr or Val
  misc_feature (28)..(28): Xaa = Asp, Glu, Phe, Gly, Ile, Lys, Gln, Arg, Ser or Val
  misc_feature (29)..(29): Xaa = Asp, Gly, His, Lys, Leu, Pro, Gln, Arg, Ser, Thr, Val or Tyr
  misc_feature (30)..(30): Xaa = Ala, Phe, Asn, Gln, Arg, Ser or Thr
  misc_feature (34)..(34): Xaa = Ala or Met
  misc_feature (35)..(35): Xaa = Gly or Met
  misc_feature (44)..(44): Xaa = Glu or Gly
  misc_feature (45)..(45): Xaa = His or Leu
  misc_feature (51)..(51): Xaa = Ile or Leu
  misc_feature (54)..(54): Xaa = Ala, Asn, Arg or Ser
  misc_feature (55)..(55): Xaa = Ala, Phe, Trp or Tyr
  misc_feature (56)..(56): Xaa = Ala, Gly or Ser
  misc_feature (58)..(58): Xaa = Glu, Gln, Ser or Thr
  misc_feature (69)..(69): Xaa = Gly or Thr
  misc_feature (75)..(75): Xaa = Ser or Thr
  misc_feature (79)..(79): Xaa = Leu or Val
  misc_feature (80)..(80): Xaa = Ala or Tyr
  misc_feature (82)..(82): Xaa = Leu or Gln
  misc_feature (87)..(87): Xaa = Lys or Arg
  misc_feature (88)..(88): Xaa = Ala or Pro
  misc_feature (93)..(93): Xaa = Ile or Val
  misc_feature (100)..(100): Xaa = Ile or Leu
  misc_feature (102)..(102): Xaa = His, Arg or Val
  misc_feature (103)..(103): Xaa = Ala, Asp, Gly, His, Leu, Asn, Arg, Ser, Thr or Val
  misc_feature (113)..(113): Xaa = Leu or Gln
QVQLVESGGGXVQXGGSLXLSCAXSXXXXXIYAXXWFRQAPGKXXEFVAGXGWXXXTXYYADSVKGRFXISRDNXKNTXXLXMNSLXXEDTAXYYCAADXDXXGFDYWGQGTXVTVSS

SEQ ID NO: 235 - protein, 25 aa, Artificial Sequence
  H-FR1 general formula 2
  misc_feature (24)..(24): Xaa = Ala or Thr
QVQLVESGGGLVQPGGSLRLSCAXS

SEQ ID NO: 236 - protein, 118 aa, Artificial Sequence
  VHH H general formula 2
  misc_feature (24)..(24): Xaa = Ala or Thr
  misc_feature (26)..(26): Xaa = Gly, His or Lys
  misc_feature (27)..(27): Xaa = Ala, Gly, Leu, Asn, Ser or Val
  misc_feature (28)..(28): Xaa = Asp, Arg or Val
  misc_feature (29)..(29): Xaa = Gly, His, Pro, Gln, Arg or Thr
  misc_feature (30)..(30): Xaa = Arg, Ser or Thr
  misc_feature (54)..(54): Xaa = Ala or Asn
  misc_feature (55)..(55): Xaa = Phe or Tyr
  misc_feature (56)..(56): Xaa = Ala or Ser
  misc_feature (58)..(58): Xaa = Glu, Gln or Thr
  misc_feature (100)..(100): Xaa = Ile or Leu
  misc_feature (102)..(102): Xaa = His or Arg
  misc_feature (103)..(103): Xaa = Ala, His or Ser
QVQLVESGGGLVQPGGSLRLSCAXSXXXXXIYAMGWFRQAPGKGLEFVAGIGWXXXTXYYADSVKGRFTISRDNTKNTLYLQMNSLRAEDTAVYYCAADXDXXGFDYWGQGTLVTVSS